European Patent Application EP 4 295 905 A1, published December 27, 2023. Title: DOSAGE AND ADMINISTRATION OF ANTI-C5 ANTIBODIES FOR TREATING PAROXYSMAL NOCTURNAL HEMOGLOBINURIA (PNH) IN PEDIATRIC PATIENTS. Applicant: ALEXION PHARMACEUTICALS, INC. Application EP 23193515.6, filed July 8, 2021. The sequence listing filed with the application follows.

SEQUENCE LISTING (50 sequences)

SEQ ID NO: 1 - protein, 10 aa, synthetic construct
GYIFSNYWIQ

SEQ ID NO: 2 - protein, 17 aa, synthetic construct
EILPGSGSTEYTENFKD

SEQ ID NO: 3 - protein, 13 aa, synthetic construct
YFFGSSPNWYFDV

SEQ ID NO: 4 - protein, 11 aa, synthetic construct
GASENIYGALN

SEQ ID NO: 5 - protein, 7 aa, synthetic construct
GATNLAD

SEQ ID NO: 6 - protein, 9 aa, synthetic construct
QNVLNTPLT

SEQ ID NO: 7 - protein, 122 aa, synthetic construct [sequence omitted]

SEQ ID NO: 8 - protein, 107 aa, synthetic construct [sequence omitted]

SEQ ID NO: 9 - protein, 326 aa, synthetic construct
ASTKGPSVFPLAPCSRSTSESTAALGCLVKDYFPEPVTVSWNSGALTSGVHTFPAVLQSSGLYSLSSVVTVPSSNFGTQTYTCNVDHKPSNTKVDKTVERKCCVECPPCPAPPVAGPSVFLFPPKPKDTLMISRTPEVTCVVVDVSQEDPEVQFNWYVDGVEVHNAKTKPREEQFNSTYRVVSVLTVLHQDWLNGKEYKCKVSNKGLPSSIEKTISKAKGQPREPQVYTLPPSQEEMTKNQVSLTCLVKGFYPSDIAVEWESNGQPENNYKTTPPVLDSDGSFFLYSRLTVDKSRWQEGNVFSCSVMHEALHNHYTQKSLSLSLGK

SEQ ID NO: 10 - protein, 447 aa, synthetic construct
QVQLVQSGAEVKKPGASVKVSCKASGYIFSNYWIQWVRQAPGQGLEWMGEILPGSGSTEYTENFKDRVTMTRDTSTSTVYMELSSLRSEDTAVYYCARYFFGSSPNWYFDVWGQGTLVTVSSASTKGPSVFPLAPCSRSTSESTAALGCLVKDYFPEPVTVSWNSGALTSGVHTFPAVLQSSGLYSLSSVVTVPSSNFGTQTYTCNVDHKPSNTKVDKTVERKCCVECPPCPAPPVAGPSVFLFPPKPKDTLMISRTPEVTCVVVDVSQEDPEVQFNWYVDGVEVHNAKTKPREEQFNSTYRVVSVLTVLHQDWLNGKEYKCKVSNKGLPSSIEKTISKAKGQPREPQVYTLPPSQEEMTNQVSLTCLVKGFYPSDIAVEWESNGQPENNYKTTPPVLDSDGSFFLYSRLTVDKSRWQEGNVFSCSVMHEALHNHYTQKSLSLSLGK

SEQ ID NO: 11 - protein, 214 aa, synthetic construct [sequence omitted]

SEQ ID NO: 12 - protein, 122 aa, synthetic construct [sequence omitted]

SEQ ID NO: 13 - protein, 326 aa, synthetic construct
ASTKGPSVFPLAPCSRSTSESTAALGCLVKDYFPEPVTVSWNSGALTSGVHTFPAVLQSSGLYSLSSVVTVPSSNFGTQTYTCNVDHKPSNTKVDKTVERKCCVECPPCPAPPVAGPSVFLFPPKPKDTLMISRTPEVTCVVVDVSQEDPEVQFNWYVDGVEVHNAKTKPREEQFNSTYRVVSVLTVLHQDWLNGKEYKCKVSNKGLPSSIEKTISKAKGQPREPQVYTLPPSQEEMTKNQVSLTCLVKGFYPSDIAVEWESNGQPENNYKTTPPVLDSDGSFFLYSRLTVDKSRWQEGNVFSCSVLHEALHSHYTQKSLSLSLGK

SEQ ID NO: 14 - protein, 448 aa, synthetic construct
QVQLVQSGAEVKKPGASVKVSCKASGHIFSNYWIQWVRQAPGQGLEWMGEILPGSGHTEYTENFKDRVTMTRDTSTSTVYMELSSLRSEDTAVYYCARYFFGSSPNWYFDVWGQGTLVTVSSASTKGPSVFPLAPCSRSTSESTAALGCLVKDYFPEPVTVSWNSGALTSGVHTFPAVLQSSGLYSLSSVVTVPSSNFGTQTYTCNVDHKPSNTKVDKTVERKCCVECPPCPAPPVAGPSVFLFPPKPKDTLMISRTPEVTCVVVDVSQEDPEVQFNWYVDGVEVHNAKTKPREEQFNSTYRVVSVLTVLHQDWLNGKEYKCKVSNKGLPSSIEKTISKAKGQPREPQVYTLPPSQEEMTKNQVSLTCLVKGFYPSDIAVEWESNGQPENNYKTTPPVLDSDGSFFLYSRLTVDKSRWQEGNVFSCSVLHEALHSHYTQKSLSLSLGK

SEQ ID NO: 15 - protein, 326 aa, synthetic construct
ASTKGPSVFPLAPCSRSTSESTAALGCLVKDYFPEPVTVSWNSGALTSGVHTFPAVLQSSGLYSLSSVVTVTSSNFGTQTYTCNVDHKPSNTKVDKTVERKCCVECPPCPAPPVAGPSVFLFPPKPKDTLYITREPEVTCVVVDVSHEDPEVQFNWYVDGMEVHNAKTKPREEQFNSTFRVVSVLTVVHQDWLNGKEYKCKVSNKGLPAPIEKTISKTKGQPREPQVYTLPPSREEMTKNQVSLTCLVKGFYPSDIAVEWESNGQPENNYKTTPPMLDSDGSFFLYSKLTVDKSRWQQGNVFSCSVMHEALHNHYTQKSLSLSPGK

SEQ ID NO: 16 - protein, 448 aa, synthetic construct
QVQLVQSGAEVKKPGASVKVSCKASGYIFSNYWIQWVRQAPGQGLEWMGEILPGSGSTEYTENFKDRVTMTRDTSTSTVYMELSSLRSEDTAVYYCARYFFGSSPNWYFDVWGQGTLVTVSSASTKGPSVFPLAPCSRSTSESTAALGCLVKDYFPEPVTVSWNSGALTSGVHTFPAVLQSSGLYSLSSVVTVTSSNFGTQTYTCNVDHKPSNTKVDKTVERKCCVECPPCPAPPVAGPSVFLFPPKPKDTLYITREPEVTCVVVDVSHEDPEVQFNWYVDGMEVHNAKTKPREEQFNSTFRVVSVLTVVHQDWLNGKEYKCKVSNKGLPAPIEKTISKTKGQPREPQVYTLPPSREEMTKNQVSLTCLVKGFYPSDIAVEWESNGQPENNYKTTPPMLDSDGSFFLYSKLTVDKSRWQQGNVFSCSVMHEALHNHYTQKSLSLSPGK

SEQ ID NO: 17 - protein, 11 aa, synthetic construct
GASENIYHALN

SEQ ID NO: 18 - protein, 17 aa, synthetic construct
EILPGSGHTEYTENFKD

SEQ ID NO: 19 - protein, 10 aa, synthetic construct
GHIFSNYWIQ

SEQ ID NO: 20 - protein, 448 aa, synthetic construct
QVQLVQSGAEVKKPGASVKVSCKASGHIFSNYWIQWVRQAPGQGLEWMGEILPGSGHTEYTENFKDRVTMTRDTSTSTVYMELSSLRSEDTAVYYCARYFFGSSPNWYFDVWGQGTLVTVSSASTKGPSVFPLAPCSRSTSESTAALGCLVKDYFPEPVTVSWNSGALTSGVHTFPAVLQSSGLYSLSSVVTVPSSNFGTQTYTCNVDHKPSNTKVDKTVERKCCVECPPCPAPPVAGPSVFLFPPKPKDTLMISRTPEVTCVVVDVSQEDPEVQFNWYVDGVEVHNAKTKPREEQFNSTYRVVSVLTVLHQDWLNGKEYKCKVSNKGLPSSIEKTISKAKGQPREPQVYTLPPSQEEMTKNQVSLTCLVKGFYPSDIAVEWESNGQPENNYKTTPPVLDSDGSFFLYSRLTVDKSRWQEGNVFSCSVMHEALHNHYTQKSLSLSLGK

SEQ ID NO: 21 - protein, 5 aa, synthetic construct
SYAIS

SEQ ID NO: 22 - protein, 17 aa, synthetic construct
GIGPFFGTANYAQKFQG

SEQ ID NO: 23 - protein, 7 aa, synthetic construct
DTPYFDY

SEQ ID NO: 24 - protein, 11 aa, synthetic construct
SGDSIPNYYVY

SEQ ID NO: 25 - protein, 7 aa, synthetic construct
DDSNRPS

SEQ ID NO: 26 - protein, 11 aa, synthetic construct
QSFDSSLNAEV

SEQ ID NO: 27 - protein, 116 aa, synthetic construct
QVQLVQSGAEVKKPGSSVKVSCKASGGTFSSYAISVWRQAPGQGLEWMGGIGPFFGTANYAQKFQGRVTITADESTSTAYMELSSLRSEDTAVYYCARDTPYFDYWGQGTLVTVSS

SEQ ID NO: 28 - protein, 108 aa, synthetic construct
DIELTQPPSVSVAPGQTARISCSGDSIPNYYVYWYQQKPGQAPVLVIYDDSNRPSGIPERFSGSNSGNTATLTISGTQAEDEADYYCQSFDSSLNAEVFGGGTKLTVL

SEQ ID NO: 29 - protein, 4 aa, synthetic construct
NYIS

SEQ ID NO: 30 - protein, 17 aa, synthetic construct
IIDPDDSYTEYSPSFQG

SEQ ID NO: 31 - protein, 8 aa, synthetic construct
YEYGGFDI

SEQ ID NO: 32 - protein, 11 aa, synthetic construct
SGDNIGNSYVH

SEQ ID NO: 33 - protein, 7 aa, synthetic construct
KDNDRPS

SEQ ID NO: 34 - protein, 9 aa, synthetic construct
GTYDIESYV

SEQ ID NO: 35 - protein, 116 aa, synthetic construct
EVQLVQSGAEVKKPGESLKISCKGSGYSFTNYISWVRQMPGKGLEWMGIIDPDDSYTEYSPSFQGQVTISADKSISTAYLQWSSLKASDTAMYYCARYEYGGFDIWGQGTLVTVSS

SEQ ID NO: 36 - protein, 106 aa, synthetic construct
SYELTQPPSVSVAPGQTARISCSGDNIGNSYVHWYQQKPGQAPVLVIYKDNDRPSGIPERFSGSNSGNTATLTISGTQAEDEADYYCGTYDIESYVFGGGTKLTVL

SEQ ID NO: 37 - protein, 6 aa, synthetic construct
SSYYVA

SEQ ID NO: 38 - protein, 17 aa, synthetic construct
AIYTGSGATYKASWAKG

SEQ ID NO: 39 - protein, 13 aa, synthetic construct
DGGYDYPTHAMHY

SEQ ID NO: 40 - protein, 11 aa, synthetic construct
QASQNIGSSLA

SEQ ID NO: 41 - protein, 7 aa, synthetic construct
GASKTHS

SEQ ID NO: 42 - protein, 12 aa, synthetic construct
QSTKVGSSYGNH

SEQ ID NO: 43 - protein, 123 aa, synthetic construct
QVQLVESGGGLVQPGGSLRLSCAASGFTSHSSYYVAWVRQAPGKGLEWVGAIYTGSGATYKASWAKGRFTISKDTSKNQVVLTMTNMDPVDTATYYCASDGGYDYPTHAMHYWGQGTLVTVSS

SEQ ID NO: 44 - protein, 110 aa, synthetic construct
DVVMTQSPSSLSASVGDRVTITCQASQNIGSSLAWYQQKPGQAPRLLIYGASKTHSGVPSRFSGSGSGTDFTLTISSLQPEDVATYYCQSTKVGSSYGNHFGGGTKVEIK

SEQ ID NO: 45 - protein, 451 aa, synthetic construct
QVQLVESGGGLVQPGRSLRLSCAASGFTVHSSYYMAWVRQAPGKGLEWVGAIFTGSGAEYKAEWAKGRVTISKDTSKNQVVLTMTNMDPVDTATYYCASDAGYDYPTHAMHYWGQGTLVTVSSASTKGPSVFPLAPSSKSTSGGTAALGCLVKDYFPEPVTVSWNSGALTSGVHTFPAVLQSSGLYSLSSVVTVPSSSLGTQTYICNVNHKPSNTKVDKKVEPKSCDKTHTCPPCPAPELRRGPKVFLFPPKPKDTLMISRTPEVTCVVVDVSHEDPEVKFNWYVDGVEVHNAKTKPREEQYNSTYRVVSVLTVLHQDWLNGKEYKCKVSNKGLPSSIEKTISKAKGQPREPQVYTLPPSREEMTKNQVSLTCLVKGFYPSDIAVEWESNGQPENNYKTTPPVLDSDGSFFLYSKLTVDKSRWQQGNVFSCSVLHEALHAHYTRKELSLSP

SEQ ID NO: 46 - protein, 217 aa, synthetic construct
DIQMTQSPSSLSASVGDRVTITCRASQGISSSLAWYQQKPGKAPKLLIYGASETESGVPSRFSGSGSGTDFTLTISSLQPEDFATYYCQNTKVGSSYGNTFGGGTKVEIKRTVAAPSVFIFPPSDEQLKSGTASVVCLLNNFYPREAKVQWKVDNALQSGNSQESVTEQDSKDSTYSLSSTLTLSKADYEKHKVYACEVTHQGLSSPVTKSFNRGEC

SEQ ID NO: 47 - protein, 120 aa, synthetic construct
QVQLQESGPGLVKPSETLSLTCTVSGDSVSSSYWTWIRQPPGKGLEWIGYIYYSGSSNYNPSLKSRATISVDTSKNQFSLKLSSVTAADTAVYYCAREGNVDTTMIFDYWGQGTLVTVSS

SEQ ID NO: 48 - protein, 107 aa, synthetic construct
AIQMTQSPSSLSASVGDRVTITCRASQGIRNDLGWYQQKPGKAPKLLIYAASSLQSGVPSRFAGRGSGTDFTLTISSLQPEDFATYYCLQDFNYPWTFGQGTKVEIK

SEQ ID NO: 49 - protein, 447 aa, synthetic construct
QVQLQESGPGLVKPSETLSLTCTVSGDSVSSSYWTWIRQPPGKGLEWIGYIYYSGSSNYNPSLKSRATISVDTSKNQFSLKLSSVTAADTAVYYCAREGNVDTTMIFDYWGQGTLVTVSSASTKGPSVFPLAPCSRSTSESTAALGCLVKDYFPEPVTVSWNSGALTSGVHTFPAVLQSSGLYSLSSVVTVPSSSLGTKTYTCNVDHKPSNTKVDKRVESKYGPPCPPCPAPEFLGGPSVFLFPPKPKDTLMISRTPEVTCVVVDVSQEDPEVQFNWYVDGVEVHNAKTKPREEQFNSTYRVVSVLTVLHQDWLNGKEYKCKVSNKGLPSSIEKTISKAKGQPREPQVYTLPPSQEEMTKNQVSLTCLVKGFYPSDIAVEWESNGQPENNYKTTPPVLDSDGSFFLYSRLTVDKSRWQEGNVFSCSVMHEALHNHYTQKSLSLSLGK

SEQ ID NO: 50 - protein, 214 aa, synthetic construct
AIQMTQSPSSLSASVGDRVTITCRASQGIRNDLGWYQQKPGKAPKLLIYAASSLQSGVPSRFAGRGSGTDFTLTISSLQPEDFATYYCLQDFNYPWTFGQGTKVEIKRTVAAPSVFIFPPSDEQLKSGTASVVCLLNNFYPREAKVQWKVDNALQSGNSQESVTEQDSKDSTYSLSSTLTLSKADYEKHKVYACEVTHQGLSSPVTKSFNRGEC